European Patent Application EP 4 378 961 A1, published June 5, 2024. Title: 一种基于全人源单域抗体的抗新型冠状病毒双特异性中和抗体及其应用. Applicant: 上海博奥明赛生物科技有限公司. The sequence listing filed with the application follows.

SEQUENCE LISTING (6 sequences)

SEQ ID NO: 1 - protein, 118 aa, artificial sequence
  source 1..118: note = n3113.4 Amino acid sequence of the variable region of the heavy chain
EVQLVESGGGLVQPGGSLRLSCAASDSSFYDYEMSWVRQVPGKTPEWIGSMYPSGRTYINPSLKSLVTISRDNSENMLYLQMNSLRAEDTAMYYCVSNWASGSTGDYWGQGTLVTVSS

SEQ ID NO: 2 - protein, 120 aa, artificial sequence
  source 1..120: note = n3130.6 Amino acid sequence of the variable region of the heavy chain
EVQLVESGGGLVQPGGSLRLSCAASDFYFDYYEMSWVRQAPGQGLEWVSTISGLGGATYYADSVKGRFTISRDNSKNTLYLQMNSLRAEDTALYYCATRSPFGDYAFSYWGQGTLVTVSS

SEQ ID NO: 3 - protein, 20 aa, artificial sequence
  source 1..20: note = Amino acid sequence of peptide adaptor
GGGGSGGGGSGGGGSGGGGS

SEQ ID NO: 4 - DNA, 354 bp, artificial sequence
  source 1..354: mol_type = other DNA; note = n3113.4 Nucleic acid sequence of the variable region of the heavy chain
gaagttcagctggttgaatctggtggtggtctggtacagccaggtggtagcctgcgtctgagctgtgcagcgagcgatagcagcttctatgactatgaaatgtcctgggtacgtcaagttccaggtaagaccccggaatggatcggcagcatgtacccgagcggccgtacttacatcaacccgtctctgaaatccctggttaccatcagccgtgataactctgaaaacatgctgtatctgcagatgaactccctgcgcgctgaagataccgcaatgtattactgcgtgagcaactgggcatccggctctaccggtgactactggggtcagggcaccctggtcactgtatcttct

SEQ ID NO: 5 - DNA, 360 bp, artificial sequence
  source 1..360: mol_type = other DNA; note = n3130.6Nucleic acid sequence of the variable region of the heavy chain
gaagtgcagctggtagaatctggcggcggtctggttcaaccaggcggttctctgcgcctgtcttgtgctgcttctgacttctactttgattactacgaaatgagctgggttcgtcaggctccaggtcagggtctggaatgggtatctactatctccggtctgggcggcgctacctattacgcggatagcgttaaaggccgtttcacgatcagccgtgacaactctaaaaacactctgtacctgcagatgaacagcctgcgtgcagaagacactgcactgtattactgtgctacccgtagcccgtttggtgattacgcgttctcctactggggccagggcactctggttaccgttagcagc

SEQ ID NO: 6 - DNA, 60 bp, artificial sequence
  source 1..60: mol_type = other DNA; note = The nucleic acid sequence of a peptide adaptor
ggtggcggtggttctggtggtggcggttctggtggtggtggttctggtggtggtggtagc